European Patent Application EP 4 644 551 A1, published November 5, 2025. Title: 2-hydroxyisoflavanone C-glycoside dehydratase gene and use thereof. Applicant: SUNTORY HOLDINGS LIMITED. The sequence listing filed with the application follows.

SEQUENCE LISTING (10 sequences)

SEQ ID NO: 1 - DNA, 347 bp, Dianthus hybrida
  source 1..347: mol_type = other DNA
tcagttcagctcacttcagttcagttcagcacagctatattatttaatagaacttcattcagttcagctcagctcaattcagttcagttcagctcatttcagttcagttcagctgtaaaaagtccgaaagaacagccatttttcgggacaggaggcagaaacccagaatcattcctaaatgaattcagcactgtagttcttctaacttcctataatacgtcatatgaaagtcaacacaagatctttgctcagaagaagggggtgatagtgaaggcgactaaagatcaaatcacagctatgacagcagaaatcgaacaagagaaagagaagaacaaatcaacgacgac

SEQ ID NO: 2 - DNA, 487 bp, Dianthus hybrida
  source 1..487: mol_type = other DNA
tcaacaggtaatatatttgtcgacattacgctcgctaatctctatatttttgtcaaaaacttgctttagatgtagctaattgaaggtacctataggattagtgtgaccctgtaagcaaatcggtttgtcgacatttttgacgcttgtctatgttcagtgtataaaaaattttcttgtgactcaatatgtgtgtgtaattttatagggtggcatgaacactccgtttattagttcaagggcaacaaagatcataatggtagtagacggtcgaggccgcctcgagatgccggccttaaacgatagcatagatggcacaaccgaaaactattacaagcaagtcagcacggaactaaagccgggtatggtgtttgtcgttcctcccggccatcctatggttctaatgtcttctcaggacgaaaaactcgaaactatttgctacgaagtgaatgccaaaggaaatcaaaagttttccatcgcagggaaagtc

SEQ ID NO: 3 - DNA, 1161 bp, Dianthus caryophyllus
  source 1..1161: mol_type = other DNA
atgggtgaaaatggaataaaaaatgagagtaacacttgttatgtgttcaatgatgaagattttagtacaatatttaagactgaagaagggaaactaagtgttcttaagaaatttggtggttttttgagaggaattgagaagtatagaatgttgatctttgagtcaaatcctctgtcttttttgacacctagttactatgattctgatatcatcttctttgtcggacatggaaaaggaacaataagtttagtatttgaaaataggagagaaagttataacattgaaaagggacatctaatgacgataccagcaggagtaacattctacattatcaacaccgacgacaaaaacaaattggtgttgtccatgtttctcatttccattacaaataccggtgactttgtgccatttttcgggacaggaggcagaaacccagaatcattcctaaatgcattcagcactgaagttcttcaaacttcctataatacgtcatatgacagtctacagaagatctttgctcagaagaagggggtaatagtgaaggcgactaaagatcaaatcacagctatgacagctgaaaacgaacaagagaaagagaagaacaaatcaacgacgacacaatttggaccgtgtcaaatctatagttatttgagggagtctaatgaatatgggaaactttttatggttgattataatgaatatcagaaacttcaagactttaacatgttcatctcctttagcaaccttcaacagggtggcatgaacactccgtttattagttcaagggcaacaaagatcataatggtagtagacggtcgaggccgcctcgagatgccggccttaaacgatagcatagatggcacaaccgaaaactattacaagcaagtcagcgcggaactaaagccgggaatggtgtttgtcgttcctcccggccatcctatggttctaatgtcttctcaggacgaaaaactcgaaactatttgctacgaagtgaatgccaaaggaaatcaaaagttttccctcgcagggaaagtgaacttgatgaagaacatacaaaaagaggcaaaggttttgtcatttggaacattagctgaagaggttgaccttgtgctcaacagtcaacagcaaaatttcttcataaaagctcctacttttaagtaa

SEQ ID NO: 4 - protein, 386 aa, Dianthus caryophyllus
MGENGIKNESNTCYVFNDEDFSTIFKTEEGKLSVLKKFGGFLRGIEKYRMLIFESNPLSFLTPSYYDSDIIFFVGHGKGTISLVFENRRESYNIEKGHLMTIPAGVTFYIINTDDKNKLVLSMFLISITNTGDFVPFFGTGGRNPESFLNAFSTEVLQTSYNTSYDSLQKIFAQKKGVIVKATKDQITAMTAENEQEKEKNKSTTTQFGPCQIYSYLRESNEYGKLFMVDYNEYQKLQDFNMFISFSNLQQGGMNTPFISSRATKIIMVVDGRGRLEMPALNDSIDGTTENYYKQVSAELKPGMVFVVPPGHPMVLMSSQDEKLETICYEVNAKGNQKFSLAGKVNLMKNIQKEAKVLSFGTLAEEVDLVLNSQQQNFFIKAPTFK

SEQ ID NO: 5 - DNA, 1155 bp, Silene littorea
  source 1..1155: mol_type = other DNA
atggctttgtcaaatggaaagggagagaatgggaagccatatgtgttcaaagatgaagattttagtacattgtttgagacccaagaagggagtttacgagttcttcagaaatttaatcaaaattctgatgttttaagaggaattcagaattataggatgttgattttcgaagcgaatccgttgagttttctaactcctagtcattgggattctgatatcattttctttgttggtcaaggaaaaggaactatcagtctggtttttgaaaagaagagagaaagcttcaacattgaaaagggacatctcatgacaataccagcaggagttacattctacattatcaacagagatgataccgataaattagtcctctcaatgtttgtcagttcgattgctaatcctggtgattttgtgccatttttcacggcaggaggcggtcaagactctgaatcattcctatctgcattcagcactgaggttcttgaagcagcttacaatgaatcaaatgaaacactaagcaagatcttttcgcaacaggggaagggggtgatagtgaaggcatccaaagagcaaattgaagctctgacagctgaagaagtgacgacggaaagcaatttcgggccttgccaaatccttagttatcttcgagagtcgagtgaatgtgggagacttttcatggttgattactgtcaatataagaaactccaagacttcaatatgttcatctccttttgcaaccttgaaccgggatgcatgaatagtccatttattagctcaagggcaacaaagatcataatggtggtaaaggggcgaggccgagttgagatggcagcctctcgccctggcgaaaagggctcaatagaaattcagtacatgaaaatcagctcggaattgaaaccgggtgtggtgtttgttattcctccagggcaccctatggtcctaatggcttctcaggattcagttttagaaactatttgctatgaagtcaatgctaaaggaaatcagaaattttcaattgcagggaaagtgaacgtgatgaagaacattcagaaagaagcaaaagtacttacatttggaaaatcagctgaagaagttgacaaggtgctcgacagttcgcagtcggattctttcttgaaagctactggtaacaagtaa

SEQ ID NO: 6 - protein, 384 aa, Silene littorea
MALSNGKGENGKPYVFKDEDFSTLFETQEGSLRVLQKFNQNSDVLRGIQNYRMLIFEANPLSFLTPSHWDSDIIFFVGQGKGTISLVFEKKRESFNIEKGHLMTIPAGVTFYIINRDDTDKLVLSMFVSSIANPGDFVPFFTAGGGQDSESFLSAFSTEVLEAAYNESNETLSKIFSQQGKGVIVKASKEQIEALTAEEVTTESNFGPCQILSYLRESSECGRLFMVDYCQYKKLQDFNMFISFCNLEPGCMNSPFISSRATKIIMVVKGRGRVEMAASRPGEKGSIEIQYMKISSELKPGVVFVIPPGHPMVLMASQDSVLETICYEVNAKGNQKFSIAGKVNVMKNIQKEAKVLTFGKSAEEVDKVLDSSQSDSFLKATGNK

SEQ ID NO: 7 - DNA, 1152 bp, Heliosperma pusillum
  source 1..1152: mol_type = other DNA
atggctttgttaaatggaaatggagagtgtgggaaaccatatgtgtttaaagatgaagattttagtacattgtttaagactgaagaaggaagtttaagtgttcttcagaaatttaatgaaagttctgatgttttaagagggattgagaattataggatgttaatctttgaagcaaatccattgagtttcttaactcctagtcattgggattctgatatcattttctttgttggtcaaggaaaaggaacaatcagcctggtttttgaaaaaaagagagaaagctttaacattgaaaagggacatctaatggttataccagctggagttacattctacattatcaacagagatgacactcataaattagtcctctcaatgtttgttagttctattgctaatcctggtgattttgcgccatttttcggtgcaggaggtcaagaccctgaatcattcctatttgcattcagcactgaggttcttgaagcagcttacaatgcatcaattaaaacactacagggcaccttttcggggaagggagtgatagtgaaggcatccaaagagcaaattaaagctctggcagctgaagaagtgacggaaagcaattttgggccatgccaaatccttagttatcttagagagtcgaatgaatgcgggagactcttcatggttgattactgtgaatataagaaactccaagacttcaatatgttcatctccttctgcaaccttgaaccgggatgcatgaatagtccatttattagttcaagggcaacaaagatcataatggtggtaaaggggcgaggtcgagtggagatggcagtttctcgcaatggcgaaaagggctcaacaggaactcaatataagaaaatcagctctgaattgaagccgggcgtagtgtttgttattcctccagggcaccctatggtccttatggcttctcaggacgaagttctagaaactatttgctatgaagtcaatgctaaaggaaatcagaagttttcacttgcaggtaaagtgaacttgatgaagaacattcagaaagaagcaaaagtactgtcatttggaacatcagctgaagaagtagacagtatgcttgacagtcagcagtcggatttctttttaaaagctactagtaacaaattacaggactag

SEQ ID NO: 8 - protein, 383 aa, Heliosperma pusillum
MALLNGNGECGKPYVFKDEDFSTLFKTEEGSLSVLQKFNESSDVLRGIENYRMLIFEANPLSFLTPSHWDSDIIFFVGQGKGTISLVFEKKRESFNIEKGHLMVIPAGVTFYIINRDDTHKLVLSMFVSSIANPGDFAPFFGAGGQDPESFLFAFSTEVLEAAYNASIKTLQGTFSGKGVIVKASKEQIKALAAEEVTESNFGPCQILSYLRESNECGRLFMVDYCEYKKLQDFNMFISFCNLEPGCMNSPFISSRATKIIMVVKGRGRVEMAVSRNGEKGSTGTQYKKISSELKPGVVFVIPPGHPMVLMASQDEVLETICYEVNAKGNQKFSLAGKVNLMKNIQKEAKVLSFGTSAEEVDSMLDSQQSDFFLKATSNKLQD

SEQ ID NO: 9 - DNA, 1158 bp, Dianthus hybrida
  source 1..1158: mol_type = other DNA
atgggtgaaaatggagtcaaaattgtgagtaacacttgttatgtgttcaatgatgaagattttagtacaatgtttaagactgaagaagggaaactaagtgttcttaagaaatttggtggttttttgagaggaattgagaagtatagaatgttgatctttgaatcaaatcctctgtcttttttgacacctagtcactatgattctgatatcatcttctttgttggacatggaaaaggaacaataagtttagtatttgaaaataggagagaaagttacaacattgaaaagggacatctaatgacgataccagcaggtgtaacattttacattatcaacaccgacgacaaaaacaaattgatgttgtccatgtttgtcatttccattacaaataccggtgactttgtgccattttttgggacaggaggtggaaacccagaatcattcctaaatgcattcagcactgaagtgcttcaaacttcctataatacgtcatatgacagtctacagaagatctttgctcagaagaagggggtgatagtgaaggcgactaaagatcaaatcacagctatgacagcagaaatcgaacaagagaaagagaagaacaaatcaacgacgacacaatttggaccgtgtcaaatctatagttatttgagggagtctaatgaatatgggaaactttttatggttgattataatgaatatcagaaacttcaagactttaacatgttcatctcctttagcaaccttcaacagggtggcatgaacactccgtttattagttcaagggcaacaaagatcataatggtagtagacggtcgaggccacctcgagatggcggccttaaatgatagcatagatggcacaaccgaaaactattacaagcaagtcagcacggaactaaagccgggtatggtgtttgtcgttcctcccggccatcctatggttctaatgtcttctcaggacgaaaaactcgaaactatttgctacgaagtgaatgccaaaggaaatcaaaagttttccctcgcagggaaagtgaacttgatgaagaacatacaaaaagaggcaaaggttttgtcatttggaacattagctgaagaggttgaccttgtgctcaacggtcaacagcaaaatttcttcataaaagctcctactttttaa

SEQ ID NO: 10 - protein, 385 aa, Dianthus hybrida
MGENGVKIVSNTCYVFNDEDFSTMFKTEEGKLSVLKKFGGFLRGIEKYRMLIFESNPLSFLTPSHYDSDIIFFVGHGKGTISLVFENRRESYNIEKGHLMTIPAGVTFYIINTDDKNKLMLSMFVISITNTGDFVPFFGTGGGNPESFLNAFSTEVLQTSYNTSYDSLQKIFAQKKGVIVKATKDQITAMTAEIEQEKEKNKSTTTQFGPCQIYSYLRESNEYGKLFMVDYNEYQKLQDFNMFISFSNLQQGGMNTPFISSRATKIIMVVDGRGHLEMAALNDSIDGTTENYYKQVSTELKPGMVFVVPPGHPMVLMSSQDEKLETICYEVNAKGNQKFSLAGKVNLMKNIQKEAKVLSFGTLAEEVDLVLNGQQQNFFIKAPTF